European Patent Application EP 4 406 968 A1, published July 31, 2024. Title: ANTI-KLB ANTIBODIES AND USES. Applicant: JIANGSU HENGRUI PHARMACEUTICALS CO., LTD. Application CN. The sequence listing filed with the application follows.

SEQUENCE LISTING (81 sequences)

SEQ ID NO: 1 - protein, 733 aa, Artificial Sequence
  DOMAIN 1..733: note = FGFR1c
MWSWKCLLFWAVLVTATLCTARPSPTLPEQDALPSSEDDDDDDDSSSEEKETDNTKPNRMPVAPYWTSPEKMEKKLHAVPAAKTVKFKCPSSGTPNPTLRWLKNGKEFKPDHRIGGYKVRYATWSIIMDSVVPSDKGNYTCIVENEYGSINHTYQLDVVERSPHRPILQAGLPANKTVALGSNVEFMCKVYSDPQPHIQWLKHIEVNGSKIGPDNLPYVQILKTAGVNTTDKEMEVLHLRNVSFEDAGEYTCLAGNSIGLSHHSAWLTVLEALEERPAVMTSPLYLEIIIYCTGAFLISCMVGSVIVYKMKSGTKKSDFHSQMAVHKLAKSIPLRRQVTVSADSSASMNSGVLLVRPSRLSSSGTPMLAGVSEYELPEDPRWELPRDRLVLGKPLGEGCFGQVVLAEAIGLDKDKPNRVTKVAVKMLKSDATEKDLSDLISEMEMMKMIGKHKNIINLLGACTQDGPLYVIVEYASKGNLREYLQARRPPGLEYCYNPSHNPEEQLSSKDLVSCAYQVARGMEYLASKKCIHRDLAARNVLVTEDNVMKIADFGLARDIHHIDYYKKTTNGRLPVKWMAPEALFDRIYTHQSDVWSFGVLLWEIFTLGGSPYPGVPVEELFKLLKEGHRMDKPSNCTNELYMMMRDCWHAVPSQRPTFKQLVEDLDRIVALTSNQEYLDLSMPLDQYSPSFPDTRSSTCSSGEDSVFSHEPLPEEPCLPRHPAQLANGGLKRR

SEQ ID NO: 2 - protein, 118 aa, Mus musculus
  DOMAIN 1..118: note = mAb-99
EVQLQQSGAELVRPGSSVKMSCKTSGYTFTNYGINWVKQRPRQGLEWIGYIYIGNGDIEYNAKFKGKATLTSDTSSSTAYMQLSSLTSEDSAIYFCARGRGLGHFDVWGTGTTVTVSS

SEQ ID NO: 3 - protein, 107 aa, Mus musculus
  DOMAIN 1..107: note = mAb-99
DVQITQSPSYLAASPGETITINCRASKSISKFLAWFQEKPGKTNKLLIYSGSTLQSGIPSRFSGSGSGTDFTLTISGLEPEDFAMYYCQQHNEYPWTFGGGTKLEIK

SEQ ID NO: 4 - protein, 115 aa, Mus musculus
  DOMAIN 1..115: note = mAb-18
QVQLQQSGPELVRPGVSVKISCKGSGYTFTDYAMHWVKQTHAKSLEWIGVISTYSGTTNYNQNFKGKATVTVDKSSSTAYMELARLTSEDSAIYYCARSGPLDYWGQGTSLTVSS

SEQ ID NO: 5 - protein, 108 aa, Mus musculus
  DOMAIN 1..108: note = mAb-18
ENVLTQSPAIMSASPGEKVTMTCRASSSVSSSYLHWYQQKSGASPKLWIYSTSNLASGVPERFSGSGSGTSYSLTISSVEAEDAATYYCQQYSGYPLTFGSGTKLEIK

SEQ ID NO: 6 - protein, 5 aa, Artificial Sequence
  DOMAIN 1..5: note = mAb-99HCDR1
NYGIN

SEQ ID NO: 7 - protein, 17 aa, Artificial Sequence
  DOMAIN 1..17: note = mAb-99HCDR2
YIYIGNGDIEYNAKFKG

SEQ ID NO: 8 - protein, 9 aa, Artificial Sequence
  DOMAIN 1..9: note = mAb-99HCDR3
GRGLGHFDV

SEQ ID NO: 9 - protein, 11 aa, Artificial Sequence
  DOMAIN 1..11: note = mAb-99LCDR1
RASKSISKFLA

SEQ ID NO: 10 - protein, 7 aa, Artificial Sequence
  DOMAIN 1..7: note = mAb-99LCDR2
SGSTLQS

SEQ ID NO: 11 - protein, 9 aa, Artificial Sequence
  DOMAIN 1..9: note = mAb-99LCDR3
QQHNEYPWT

SEQ ID NO: 12 - protein, 5 aa, Artificial Sequence
  DOMAIN 1..5: note = mAb-18HCDR1
DYAMH

SEQ ID NO: 13 - protein, 17 aa, Artificial Sequence
  DOMAIN 1..17: note = mAb-18HCDR2
VISTYSGTTNYNQNFKG

SEQ ID NO: 14 - protein, 6 aa, Artificial Sequence
  DOMAIN 1..6: note = mAb-18HCDR3
SGPLDY

SEQ ID NO: 15 - protein, 12 aa, Artificial Sequence
  DOMAIN 1..12: note = mAb-18LCDR1
RASSSVSSSYLH

SEQ ID NO: 16 - protein, 7 aa, Artificial Sequence
  DOMAIN 1..7: note = mAb-18LCDR2
STSNLAS

SEQ ID NO: 17 - protein, 9 aa, Artificial Sequence
  DOMAIN 1..9: note = mAb-18LCDR3
QQYSGYPLT

SEQ ID NO: 18 - protein, 120 aa, Artificial Sequence
  DOMAIN 1..120: note = hAb-23
QVQLVQSGAEVKKPGSSVKVSCKASGGTFSSYAISWVRQAPGQGLEWMGGIIPIFGTANYAQKFQGRVTITADESTSTAYMELSSLRSEDTAVYYCARELVSYYYGMDVWGQGTMVTVSS

SEQ ID NO: 19 - protein, 107 aa, Artificial Sequence
  DOMAIN 1..107: note = hAb-23
DIVMTQSPSSLSASVGDRVTITCQASQDISNYLNWYQQKPGKAPKLLIYDASNLETGVPSRFSGSGSGTDFTFTISSLQPEDIATYYCQQYDNLPLTFGGGTKVEIK

SEQ ID NO: 20 - protein, 450 aa, Artificial Sequence
  CHAIN 1..450: note = hAb-23
QVQLVQSGAEVKKPGSSVKVSCKASGGTFSSYAISWVRQAPGQGLEWMGGIIPIFGTANYAQKFQGRVTITADESTSTAYMELSSLRSEDTAVYYCARELVSYYYGMDVWGQGTMVTVSSASTKGPSVFPLAPSSKSTSGGTAALGCLVKDYFPEPVTVSWNSGALTSGVHTFPAVLQSSGLYSLSSVVTVPSSSLGTQTYICNVNHKPSNTKVDKKVEPKSCDKTHTCPPCPAPEAAGGPSVFLFPPKPKDTLMISRTPEVTCVVVDVSHEDPEVKFNWYVDGVEVHNAKTKPREEQYNSTYRVVSVLTVLHQDWLNGKEYKCKVSNKALPAPIEKTISKAKGQPREPQVYTLPPSRDELTKNQVSLTCLVKGFYPSDIAVEWESNGQPENNYKTTPPVLDSDGSFFLYSKLTVDKSRWQQGNVFSCSVMHEALHNHYTQKSLSLSPGK

SEQ ID NO: 21 - protein, 214 aa, Artificial Sequence
  CHAIN 1..214: note = hAb-23
DIVMTQSPSSLSASVGDRVTITCQASQDISNYLNWYQQKPGKAPKLLIYDASNLETGVPSRFSGSGSGTDFTFTISSLQPEDIATYYCQQYDNLPLTFGGGTKVEIKRTVAAPSVFIFPPSDEQLKSGTASVVCLLNNFYPREAKVQWKVDNALQSGNSQESVTEQDSKDSTYSLSSTLTLSKADYEKHKVYACEVTHQGLSSPVTKSFNRGEC

SEQ ID NO: 22 - protein, 330 aa, Artificial Sequence
  DOMAIN 1..330: note = IgG1L234AL235A
ASTKGPSVFPLAPSSKSTSGGTAALGCLVKDYFPEPVTVSWNSGALTSGVHTFPAVLQSSGLYSLSSVVTVPSSSLGTQTYICNVNHKPSNTKVDKKVEPKSCDKTHTCPPCPAPEAAGGPSVFLFPPKPKDTLMISRTPEVTCVVVDVSHEDPEVKFNWYVDGVEVHNAKTKPREEQYNSTYRVVSVLTVLHQDWLNGKEYKCKVSNKALPAPIEKTISKAKGQPREPQVYTLPPSRDELTKNQVSLTCLVKGFYPSDIAVEWESNGQPENNYKTTPPVLDSDGSFFLYSKLTVDKSRWQQGNVFSCSVMHEALHNHYTQKSLSLSPGK

SEQ ID NO: 23 - protein, 107 aa, Artificial Sequence [sequence omitted]

SEQ ID NO: 24 - protein, 5 aa, Artificial Sequence
  DOMAIN 1..5: note = hAb-23HCDR1
SYAIS

SEQ ID NO: 25 - protein, 17 aa, Artificial Sequence
  DOMAIN 1..17: note = hAb-23HCDR2
GIIPIFGTANYAQKFQG

SEQ ID NO: 26 - protein, 11 aa, Artificial Sequence
  DOMAIN 1..11: note = hAb-23HCDR3
ELVSYYYGMDV

SEQ ID NO: 27 - protein, 11 aa, Artificial Sequence
  DOMAIN 1..11: note = hAb-23LCDR1
QASQDISNYLN

SEQ ID NO: 28 - protein, 7 aa, Artificial Sequence
  DOMAIN 1..7: note = hAb-23LCDR2
DASNLET

SEQ ID NO: 29 - protein, 9 aa, Artificial Sequence
  DOMAIN 1..9: note = hAb-23LCDR3
QQYDNLPLT

SEQ ID NO: 30 - protein, 118 aa, Artificial Sequence
  DOMAIN 1..118: note = hAb99VH1
EVQLVQSGAEVKKPGASVKVSCKASGYTFTNYGINWVRQAPGQRLEWMGYIYIGNGDIEYNAKFKGRVTITSDTSASTAYMELSSLRSEDTAVYYCARGRGLGHFDVWGQGTTVTVSS

SEQ ID NO: 31 - protein, 118 aa, Artificial Sequence
  DOMAIN 1..118: note = hAb99VH2
EVQLVQSGAEVKKPGASVKVSCKASGYTFTNYGINWVRQAPGQGLEWMGYIYIGNGDIEYNAKFKGRVTITSDTSASTAYMELSSLRSEDTAVYYCARGRGLGHFDVWGQGTTVTVSS

SEQ ID NO: 32 - protein, 118 aa, Artificial Sequence
  DOMAIN 1..118: note = hAb99VH3
EVQLVQSGAEVKKPGASVKVSCKTSGYTFTNYGINWVRQAPGQGLEWMGYIYIGNGDIEYNAKFKGRVTITSDTSASTAYMELSSLRSEDTAVYFCARGRGLGHFDVWGQGTTVTVSS

SEQ ID NO: 33 - protein, 107 aa, Artificial Sequence
  DOMAIN 1..107: note = hAb99VL1
DIQMTQSPSSLSASVGDRVTITCRASKSISKFLAWYQQKPGKANKLLIYSGSTLQSGVPSRFSGSGSGTDFTLTISSLQPEDFATYYCQQHNEYPWTFGGGTKVEIK

SEQ ID NO: 34 - protein, 107 aa, Artificial Sequence
  DOMAIN 1..107: note = hAb99VL2
DIQMTQSPSSLSASVGDRVTITCRASKSISKFLAWFQQKPGKTNKLLIYSGSTLQSGVPSRFSGSGSGTDFTLTISSLQPEDFATYYCQQHNEYPWTFGGGTKVEIK

SEQ ID NO: 35 - protein, 107 aa, Artificial Sequence
  DOMAIN 1..107: note = hAb99VL3
DVQITQSPSSLSASVGDRVTITCRASKSISKFLAWFQQKPGKTNKLLIYSGSTLQSGVPSRFSGSGSGTDFTLTISSLQPEDFATYYCQQHNEYPWTFGGGTKVEIK

SEQ ID NO: 36 - protein, 107 aa, Artificial Sequence
  DOMAIN 1..107: note = hAb99VL4
DVQITQSPSSLSASVGDRVTITCRASKSISKFLAWFQEKPGKTNKLLIYSGSTLQSGIPSRFSGSGSGTDFTLTISSLQPEDFATYYCQQHNEYPWTFGGGTKVEIK

SEQ ID NO: 37 - protein, 17 aa, Artificial Sequence
  DOMAIN 1..17: note = hAb99VH1-NV/hAb99VH2-NV/hAb99VH3-NVHCDR2
YIYIGNVDIEYNAKFKG

SEQ ID NO: 38 - protein, 17 aa, Artificial Sequence
  DOMAIN 1..17: note = hAb99VH1-NL/hAb99VH2-NL/hAb99VH3-NLHCDR2
YIYIGNLDIEYNAKFKG

SEQ ID NO: 39 - protein, 17 aa, Artificial Sequence
  DOMAIN 1..17: note = hAb99VH1-QG/hAb99VH2-QG/hAb99VH3-QGHCDR2
YIYIGQGDIEYNAKFKG

SEQ ID NO: 40 - protein, 118 aa, Artificial Sequence
  DOMAIN 1..118: note = hAb99VH1-NV
EVQLVQSGAEVKKPGASVKVSCKASGYTFTNYGINWVRQAPGQRLEWMGYIYIGNVDIEYNAKFKGRVTITSDTSASTAYMELSSLRSEDTAVYYCARGRGLGHFDVWGQGTTVTVSS

SEQ ID NO: 41 - protein, 118 aa, Artificial Sequence
  DOMAIN 1..118: note = hAb99VH2-NV
EVQLVQSGAEVKKPGASVKVSCKASGYTFTNYGINWVRQAPGQGLEWMGYIYIGNVDIEYNAKFKGRVTITSDTSASTAYMELSSLRSEDTAVYYCARGRGLGHFDVWGQGTTVTVSS

SEQ ID NO: 42 - protein, 118 aa, Artificial Sequence
  DOMAIN 1..118: note = hAb99VH3-NV
EVQLVQSGAEVKKPGASVKVSCKTSGYTFTNYGINWVRQAPGQGLEWMGYIYIGNVDIEYNAKFKGRVTITSDTSASTAYMELSSLRSEDTAVYFCARGRGLGHFDVWGQGTTVTVSS

SEQ ID NO: 43 - protein, 118 aa, Artificial Sequence
  DOMAIN 1..118: note = hAb99VH1-NL
EVQLVQSGAEVKKPGASVKVSCKASGYTFTNYGINWVRQAPGQRLEWMGYIYIGNLDIEYNAKFKGRVTITSDTSASTAYMELSSLRSEDTAVYYCARGRGLGHFDVWGQGTTVTVSS

SEQ ID NO: 44 - protein, 118 aa, Artificial Sequence
  DOMAIN 1..118: note = hAb99VH2-NL
EVQLVQSGAEVKKPGASVKVSCKASGYTFTNYGINWVRQAPGQGLEWMGYIYIGNLDIEYNAKFKGRVTITSDTSASTAYMELSSLRSEDTAVYYCARGRGLGHFDVWGQGTTVTVSS

SEQ ID NO: 45 - protein, 118 aa, Artificial Sequence
  DOMAIN 1..118: note = hAb99VH3-NL
EVQLVQSGAEVKKPGASVKVSCKTSGYTFTNYGINWVRQAPGQGLEWMGYIYIGNLDIEYNAKFKGRVTITSDTSASTAYMELSSLRSEDTAVYFCARGRGLGHFDVWGQGTTVTVSS

SEQ ID NO: 46 - protein, 118 aa, Artificial Sequence
  DOMAIN 1..118: note = hAb99VH1- QG
EVQLVQSGAEVKKPGASVKVSCKASGYTFTNYGINWVRQAPGQRLEWMGYIYIGQGDIEYNAKFKGRVTITSDTSASTAYMELSSLRSEDTAVYYCARGRGLGHFDVWGQGTTVTVSS

SEQ ID NO: 47 - protein, 118 aa, Artificial Sequence
  DOMAIN 1..118: note = hAb99VH2- QG
EVQLVQSGAEVKKPGASVKVSCKASGYTFTNYGINWVRQAPGQGLEWMGYIYIGQGDIEYNAKFKGRVTITSDTSASTAYMELSSLRSEDTAVYYCARGRGLGHFDVWGQGTTVTVSS

SEQ ID NO: 48 - protein, 118 aa, Artificial Sequence
  DOMAIN 1..118: note = hAb99VH3- QG
EVQLVQSGAEVKKPGASVKVSCKTSGYTFTNYGINWVRQAPGQGLEWMGYIYIGQGDIEYNAKFKGRVTITSDTSASTAYMELSSLRSEDTAVYFCARGRGLGHFDVWGQGTTVTVSS

SEQ ID NO: 49 - protein, 115 aa, Artificial Sequence
  DOMAIN 1..115: note = hAb18VH1
EVQLVQSGAEVKKPGASVKVSCKASGYTFTDYAMHWVRQAPGQRLEWMGVISTYSGTTNYNQNFKGRVTITVDKSASTAYMELSSLRSEDTAVYYCARSGPLDYWGQGTTVTVSS

SEQ ID NO: 50 - protein, 115 aa, Artificial Sequence
  DOMAIN 1..115: note = hAb18VH2
EVQLVQSGAEVKKPGASVKVSCKGSGYTFTDYAMHWVRQAPGQRLEWMGVISTYSGTTNYNQNFKGRVTVTVDKSASTAYMELSSLRSEDTAVYYCARSGPLDYWGQGTTVTVSS

SEQ ID NO: 51 - protein, 115 aa, Artificial Sequence
  DOMAIN 1..115: note = hAb18VH3
EVQLVQSGAEVKKPGASVKVSCKGSGYTFTDYAMHWVRQAPGQRLEWIGVISTYSGTTNYNQNFKGRATVTVDKSASTAYMELSSLRSEDTAVYYCARSGPLDYWGQGTTVTVSS

SEQ ID NO: 52 - protein, 108 aa, Artificial Sequence
  DOMAIN 1..108: note = hAb18VL1
EIVLTQSPDFQSVTPKEKVTITCRASSSVSSSYLHWYQQKPDQSPKLWIYSTSNLASGVPSRFSGSGSGTDFTLTINSLEAEDAATYYCQQYSGYPLTFGQGTKLEIK

SEQ ID NO: 53 - protein, 108 aa, Artificial Sequence
  DOMAIN 1..108: note = hAb18VL2
ENVLTQSPDFQSVTPKEKVTITCRASSSVSSSYLHWYQQKPDQSPKLWIYSTSNLASGVPSRFSGSGSGTDYTLTINSLEAEDAATYYCQQYSGYPLTFGQGTKLEIK

SEQ ID NO: 54 - protein, 106 aa, Artificial Sequence
  DOMAIN 1..106: note = hAb18VL3
EIVLTQSPATLSLSPGERATLSCRASSSVSSSYLHWYQQKPGQAPKLWIYSTSNLASGVPARFSGSGSGTDFTLTISRLEPEDFAVYQQYSGYPLTFGQGTKLEIK

SEQ ID NO: 55 - protein, 106 aa, Artificial Sequence
  DOMAIN 1..106: note = hAb18VL4
ENVLTQSPATLSLSPGERATLSCRASSSVSSSYLHWYQQKPGQAPKLWIYSTSNLASGVPARFSGSGSGTDYTLTISRLEPEDFAVYQQYSGYPLTFGQGTKLEIK

SEQ ID NO: 56 - protein, 108 aa, Artificial Sequence
  DOMAIN 1..108: note = hAb18VL2-1
ENVLTQSPDFQSVTPKEKVTITCRASSSVSSSYLHWYQQKPDQSPKLWIYSTSQLASGVPSRFSGSGSGTDYTLTINSLEAEDAATYYCQQYSGYPLTFGQGTKLEIK

SEQ ID NO: 57 - protein, 108 aa, Artificial Sequence
  DOMAIN 1..108: note = hAb18VL2-2
ENVLTQSPDFQSVTPKEKVTITCRATSSVSSSYLHWYQQKPDQSPKLWIYSTSQLASGVPSRFSGSGSGTDYTLTINSLEAEDAATYYCQQYSGYPLTFGQGTKLEIK

SEQ ID NO: 58 - protein, 108 aa, Artificial Sequence
  DOMAIN 1..108: note = hAb18VL2-3
ENVLTQSPDFQSVTPKEKVTITCRVSSSVSSSYLHWYQQKPDQSPKLWIYSTSQLASGVPSRFSGSGSGTDYTLTINSLEAEDAATYYCQQYSGYPLTFGQGTKLEIK

SEQ ID NO: 59 - protein, 108 aa, Artificial Sequence
  DOMAIN 1..108: note = hAb18VL2-4
ENVLTQSPDFQSVTPKEKVTITCRASSSVSTSYLHWYQQKPDQSPKLWIYSTSQLASGVPSRFSGSGSGTDYTLTINSLEAEDAATYYCQQYSGYPLTFGQGTKLEIK

SEQ ID NO: 60 - protein, 108 aa, Artificial Sequence
  DOMAIN 1..108: note = hAb18VL2-5
ENVLTQSPDFQSVTPKEKVTITCRASSSVTSSYLHWYQQKPDQSPKLWIYSTSQLASGVPSRFSGSGSGTDYTLTINSLEAEDAATYYCQQYSGYPLTFGQGTKLEIK

SEQ ID NO: 61 - protein, 108 aa, Artificial Sequence
  DOMAIN 1..108: note = hAb18VL2-6
ENVLTQSPDFQSVTPKEKVTITCRASSSLSSSYLHWYQQKPDQSPKLWIYSTSQLASGVPSRFSGSGSGTDYTLTINSLEAEDAATYYCQQYSGYPLTFGQGTKLEIK

SEQ ID NO: 62 - protein, 108 aa, Artificial Sequence
  DOMAIN 1..108: note = hAb18VL2-7
ENVLTQSPDFQSVTPKEKVTITCRASSNVSSSYLHWYQQKPDQSPKLWIYSTSQLASGVPSRFSGSGSGTDYTLTINSLEAEDAATYYCQQYSGYPLTFGQGTKLEIK

SEQ ID NO: 63 - protein, 108 aa, Artificial Sequence
  DOMAIN 1..108: note = hAb18VL2-8
ENVLTQSPDFQSVTPKEKVTITCRATSSVSSSYLHWYQQKPDQSPKLWIYSTSNLASGVPSRFSGSGSGTDYTLTINSLEAEDAATYYCQQYSGYPLTFGQGTKLEIK

SEQ ID NO: 64 - protein, 108 aa, Artificial Sequence
  DOMAIN 1..108: note = hAb18VL2-9
ENVLTQSPDFQSVTPKEKVTITCRVSSSVSSSYLHWYQQKPDQSPKLWIYSTSNLASGVPSRFSGSGSGTDYTLTINSLEAEDAATYYCQQYSGYPLTFGQGTKLEIK

SEQ ID NO: 65 - protein, 108 aa, Artificial Sequence
  DOMAIN 1..108: note = hAb18VL2-10
ENVLTQSPDFQSVTPKEKVTITCRASSSVSTSYLHWYQQKPDQSPKLWIYSTSNLASGVPSRFSGSGSGTDYTLTINSLEAEDAATYYCQQYSGYPLTFGQGTKLEIK

SEQ ID NO: 66 - protein, 108 aa, Artificial Sequence
  DOMAIN 1..108: note = hAb18VL2-11
ENVLTQSPDFQSVTPKEKVTITCRASSSVTSSYLHWYQQKPDQSPKLWIYSTSNLASGVPSRFSGSGSGTDYTLTINSLEAEDAATYYCQQYSGYPLTFGQGTKLEIK

SEQ ID NO: 67 - protein, 108 aa, Artificial Sequence
  DOMAIN 1..108: note = hAb18VL2-12
ENVLTQSPDFQSVTPKEKVTITCRASSSLSSSYLHWYQQKPDQSPKLWIYSTSNLASGVPSRFSGSGSGTDYTLTINSLEAEDAATYYCQQYSGYPLTFGQGTKLEIK

SEQ ID NO: 68 - protein, 108 aa, Artificial Sequence
  DOMAIN 1..108: note = hAb18VL2-13
ENVLTQSPDFQSVTPKEKVTITCRASSNVSSSYLHWYQQKPDQSPKLWIYSTSNLASGVPSRFSGSGSGTDYTLTINSLEAEDAATYYCQQYSGYPLTFGQGTKLEIK

SEQ ID NO: 69 - protein, 12 aa, Artificial Sequence
  DOMAIN 1..12: note = hAb18VL2-2/hAb18VL2-8LCDR1
RATSSVSSSYLH

SEQ ID NO: 70 - protein, 12 aa, Artificial Sequence
  DOMAIN 1..12: note = hAb18VL2-3/hAb18VL2-9LCDR1
RVSSSVSSSYLH

SEQ ID NO: 71 - protein, 12 aa, Artificial Sequence
  DOMAIN 1..12: note = hAb18VL2-4/hAb18VL2-10LCDR1
RASSSVSTSYLH

SEQ ID NO: 72 - protein, 12 aa, Artificial Sequence
  DOMAIN 1..12: note = hAb18VL2-5/hAb18VL2-11LCDR1
RASSSVTSSYLH

SEQ ID NO: 73 - protein, 12 aa, Artificial Sequence
  DOMAIN 1..12: note = hAb18VL2-6/hAb18VL2-12LCDR1
RASSSLSSSYLH

SEQ ID NO: 74 - protein, 12 aa, Artificial Sequence
  DOMAIN 1..12: note = hAb18VL2-7/hAb18VL2-13LCDR1
RASSNVSSSYLH

SEQ ID NO: 75 - protein, 7 aa, Artificial Sequence
  DOMAIN 1..7: note = hAb18VL2-1/hAb18VL2-2/hAb18VL2-3/hAb18VL2-4/hAb18VL2-5/hAb18VL2-6/hAb18VL2-7LCDR2
STSQLAS

SEQ ID NO: 76 - protein, 187 aa, Artificial Sequence
  DOMAIN 1..187: note = FGF21
HHHHHHHPIPDSSPLLQFGGQVRQRYLYTDDAQQTEAHLEIREDGTVGGAADQSPESLLQLKALKPGVIQILGVKTSRFLCQRPDGALYGSLHFDPEACSFRELLLEDGYNVYQSEAHGLPLHLPGNKSPHRDPAPRGPARFLPLPGLPPALPEPPGILAPQPPDVGSSDPLSMVGPSQGRSPSYAS

SEQ ID NO: 77 - protein, 198 aa, Artificial Sequence
  DOMAIN 1..198: note = FGF19
HHHHHHLAFSDAGPHVHYGWGDPIRLRHLYTSGPHGLSSCFLRIRADGVVDCARGQSAHSLLEIKAVALRTVAIKGVHSVRYLCMGADGKMQGLLQYSEEDCAFEEEIRPDGYNVYRSEKHRLPVSLSSAKQRQLYKNRGFLPLSHFLPMLPMVPEEPEDLRGHLESDMFSSPLETDSMDPFGLVTGLEAVRSPSFEK

SEQ ID NO: 78 - protein, 448 aa, Artificial Sequence
  CHAIN 1..448: note = hAb99-13
EVQLVQSGAEVKKPGASVKVSCKASGYTFTNYGINWVRQAPGQRLEWMGYIYIGNVDIEYNAKFKGRVTITSDTSASTAYMELSSLRSEDTAVYYCARGRGLGHFDVWGQGTTVTVSSASTKGPSVFPLAPSSKSTSGGTAALGCLVKDYFPEPVTVSWNSGALTSGVHTFPAVLQSSGLYSLSSVVTVPSSSLGTQTYICNVNHKPSNTKVDKKVEPKSCDKTHTCPPCPAPEAAGGPSVFLFPPKPKDTLMISRTPEVTCVVVDVSHEDPEVKFNWYVDGVEVHNAKTKPREEQYNSTYRVVSVLTVLHQDWLNGKEYKCKVSNKALPAPIEKTISKAKGQPREPQVYTLPPSRDELTKNQVSLTCLVKGFYPSDIAVEWESNGQPENNYKTTPPVLDSDGSFFLYSKLTVDKSRWQQGNVFSCSVMHEALHNHYTQKSLSLSPGK

SEQ ID NO: 79 - protein, 214 aa, Artificial Sequence
  CHAIN 1..214: note = hAb99-13
DIQMTQSPSSLSASVGDRVTITCRASKSISKFLAWFQQKPGKTNKLLIYSGSTLQSGVPSRFSGSGSGTDFTLTISSLQPEDFATYYCQQHNEYPWTFGGGTKVEIKRTVAAPSVFIFPPSDEQLKSGTASVVCLLNNFYPREAKVQWKVDNALQSGNSQESVTEQDSKDSTYSLSSTLTLSKADYEKHKVYACEVTHQGLSSPVTKSFNRGEC

SEQ ID NO: 80 - protein, 445 aa, Artificial Sequence
  CHAIN 1..445: note = hAb18-8
EVQLVQSGAEVKKPGASVKVSCKASGYTFTDYAMHWVRQAPGQRLEWMGVISTYSGTTNYNQNFKGRVTITVDKSASTAYMELSSLRSEDTAVYYCARSGPLDYWGQGTTVTVSSASTKGPSVFPLAPSSKSTSGGTAALGCLVKDYFPEPVTVSWNSGALTSGVHTFPAVLQSSGLYSLSSVVTVPSSSLGTQTYICNVNHKPSNTKVDKKVEPKSCDKTHTCPPCPAPEAAGGPSVFLFPPKPKDTLMISRTPEVTCVVVDVSHEDPEVKFNWYVDGVEVHNAKTKPREEQYNSTYRVVSVLTVLHQDWLNGKEYKCKVSNKALPAPIEKTISKAKGQPREPQVYTLPPSRDELTKNQVSLTCLVKGFYPSDIAVEWESNGQPENNYKTTPPVLDSDGSFFLYSKLTVDKSRWQQGNVFSCSVMHEALHNHYTQKSLSLSPGK

SEQ ID NO: 81 - protein, 215 aa, Artificial Sequence
  CHAIN 1..215: note = hAb18-8
ENVLTQSPDFQSVTPKEKVTITCRATSSVSSSYLHWYQQKPDQSPKLWIYSTSQLASGVPSRFSGSGSGTDYTLTINSLEAEDAATYYCQQYSGYPLTFGQGTKLEIKRTVAAPSVFIFPPSDEQLKSGTASVVCLLNNFYPREAKVQWKVDNALQSGNSQESVTEQDSKDSTYSLSSTLTLSKADYEKHKVYACEVTHQGLSSPVTKSFNRGEC